European Patent Application EP 4 133 936 A1, published February 15, 2023. Title: A method for producing oats having high-content avenanthramides using elicitors. Applicant: KOREA RESEARCH INSTITUTE OF BIOSCIENCE AND BIOTECHNOLOGY. The sequence listing filed with the application follows.

SEQUENCE LISTING (12 sequences)

SEQ ID NO: 1 - DNA, 20 bp, Artificial Sequence
  AsPAL-F
cgatcatggagcacattctg

SEQ ID NO: 2 - DNA, 20 bp, Artificial Sequence
  AsPAL-R
tcgatgacggggttatcatt

SEQ ID NO: 3 - DNA, 20 bp, Artificial Sequence
  AsHHT1-F
ggagaagttccggaagatga

SEQ ID NO: 4 - DNA, 20 bp, Artificial Sequence
  AsHHT1-F
agaagggggaattttgcagt

SEQ ID NO: 5 - DNA, 20 bp, Artificial Sequence
  AsHHT2-F
ggagaagttccggaagatga

SEQ ID NO: 6 - DNA, 20 bp, Artificial Sequence
  AsHHT2-R
caaagtggcaggaaagaagg

SEQ ID NO: 7 - DNA, 20 bp, Artificial Sequence
  AsHHT3-F
ggagaagttccggaagatga

SEQ ID NO: 8 - DNA, 20 bp, Artificial Sequence
  AsHHT3-R
gaaagaagggggaattttgc

SEQ ID NO: 9 - DNA, 20 bp, Artificial Sequence
  AsHHT4-F
agcccaccaagctgtactgt

SEQ ID NO: 10 - DNA, 20 bp, Artificial Sequence
  AsHHT4-R
ggaccaatgctgacaaatcc

SEQ ID NO: 11 - DNA, 20 bp, Artificial Sequence
  AsActin-F
gctgtgctttccctctatgc

SEQ ID NO: 12 - DNA, 20 bp, Artificial Sequence
  AsActin-R
cgagcttctccttgatgtcc